European Patent Specification EP 3 472 337 B1, published August 16, 2023. Title: METHOD FOR PRODUCING FRUCTOSE FROM GLUCOSE OBTAINED FROM LIGNOCELLULOSIC BIOMASS. Applicant: Metgen OY. The sequence listing filed with the application follows.

SEQUENCE LISTING (7 sequences)

SEQ ID NO: 1 - protein, 368 aa, Dictyoglomus thermophilum
MPFVDHRAQKIRRSKEELLKHMQTFKLDLKFSVGIWYFTPGGGRFHEPYVEQKSIPERIEMAAEMAKFGVKGIEAHYPAEVNEENLHLYKQLEKEAGIRLVAVPLSLFYDKIFEFGSLSNPYEKYRKVAYERLVNGLKLVKEANADICIIWPGIDGYTYSYGHLYYHMWDTFEELVAQAMDEVPGVQVAIEPKPYEPAPNNIYRTTADGILAARDIEARLKNPENLKLLQEGHALVGLNPEVGHVRMGFEDLPYAYARVAREGRLFHTHWNSQPLGNYDQDLNIGVVDWDSTEALLYTLKMVGYQGYFGIDINPERMPVIKAIEINTKVLQIMNERIERLPHDRIIECYFDPENHRGELELILAENHK

SEQ ID NO: 2 - protein, 368 aa, Dictyoglomus turgidum
MPFVDHRNQKIRRSKEELLKHMQTFKLDLKFSVGIWYFTPGGGRFHEPYVEQKGIPERIEMAAEMAKYGVKGIEAHYPAEVNEENLHLYKQLEKETGIRLVAVPLSLFYDKIFEFGSLSNPYEKYRKIAYERLVNGLKLVKEANADICIIWPGIDGYTYSYGHLYYHMWDTFEELVAQAMDEVPGVQVAIEPKPYEPAPNNIYRTTADGILAARDIEARLKNPENLKLLQEGHALVGLNPEVGHVRMGFEDLPYAYARVAREGRLFHTHWNSQPLGNYDQDLNIGVVDWDSTEALLYTLKMVGYQGYFGIDINPERIPVVKAIEINTKVLQIMNERIERLPHDRIIECYFDPENHRGELELILAENHR

SEQ ID NO: 3 - protein, 444 aa, Thermotoga Neapolitana
MAEFFPEIPKVQFEGKESTNPLAFKFYDPEEIIDGKPLKDHLKFSVAFWHTFVNEGRDPFGDPTADRPWNRYTDPMDKAFARVDALFEFCEKLNIEYFCFHDRDIAPEGKTLRETNKILDKVVERIKERMKDSNVKLLWGTANLFSHPRYMHGAATTCSADVFAYAAAQVKKALEITKELGGEGYVFWGGREGYETLLNTDLGFELENLARFLRMAVDYAKRIGFTGQFLIEPKPKEPTKHQYDFDVATAYAFLKSHGLDEYFKFNIEANHATLAGHTFQHELRMARILGKLGSIDANQGDLLLGWDTDQFPTNVYDTTLAMYEVIKAGGFTKGGLNFDAKVRRASYKVEDLFIGHIAGMDTFALGFKVAYKLVKDGVLDKFIEEKYRSFREGIGRDIVEGKVDFEKLEEYIIDKETIELPSGKQEYLESLINSYIVKTILELR

SEQ ID NO: 4 - DNA, 1107 bp, Dictyoglomus thermophilum
atgccgtttgttgatcatcgtgcacagaaaattcgtcgcagcaaagaagaactgctgaaacatatgcagaccttcaaactggatctgaaatttagcgtgggcatctggtattttacaccgggtggtggtcgttttcatgaaccgtatgttgaacagaaaagcattccggaacgtattgaaatggcagcagaaatggcaaaatttggcgtgaaaggtattgaagcacattatccggctgaagtgaatgaagaaaatctgcacctgtataaacagctggaaaaagaagcaggtattcgtctggttgcagttccgctgagcctgttttatgataaaatctttgaatttggcagcctgagcaacccgtatgaaaaatatcgtaaagttgcctatgaacgcctggtgaatggtctgaaactggttaaagaagcaaacgccgatatttgcattatttggcctggtattgatggctatacctatagctatggtcacctgtattatcacatgtgggatacctttgaagaactggttgcacaggcaatggatgaagttccgggtgttcaggttgcaattgaaccgaaaccgtatgaaccggcaccgaataacatttatcgtaccaccgcagatggtattctggcagcacgtgatattgaagcgcgtctgaaaaatccggaaaacctgaaactgctgcaagaaggtcacgcactggttggtctgaatccggaagttggtcatgttcgtatgggttttgaagatctgccgtatgcatatgcccgtgttgcacgtgaaggtcgtctgtttcatacccattggaatagccagccgctgggtaattatgatcaggatctgaatattggtgtggtggattgggatagcaccgaagcactgctgtataccctgaaaatggttggttatcagggctattttggcatcgatatcaatccggaacgcatgccggttattaaagccattgaaattaacaccaaagtgctgcagattatgaacgaacgcattgaacgtctgccgcatgatcgtattattgagtgttattttgaccctgagaatcatcgtggtgaactggaactgattctggccgaaaatcataaataa

SEQ ID NO: 5 - DNA, 1107 bp, Dictyoglomus turgidum
atgccgtttgtggatcatcgtaatcagaaaattcgtcgcagcaaagaagaactgctgaaacatatgcagaccttcaaactggatctgaaatttagcgtgggcatctggtattttacaccgggtggtggtcgttttcatgaaccgtatgttgaacagaaaggtattccggaacgtattgaaatggcagcagaaatggcaaaatatggcgttaaaggtatcgaagcacattatccggctgaagtgaatgaagaaaatctgcacctgtataaacagctggaaaaagaaaccggtattcgtctggttgcagttccgctgagcctgttttatgataaaatctttgaatttggcagcctgagcaacccgtatgaaaaatatcgtaaaattgcctatgaacgcctggtgaatggtctgaaactggttaaagaagcaaacgccgatatttgcattatttggcctggtattgatggctatacctatagctatggtcacctgtattatcacatgtgggatacctttgaagaactggttgcacaggcaatggatgaagttccgggtgttcaggttgcaattgaaccgaaaccgtatgaaccggcaccgaataacatttatcgtaccaccgcagatggtattctggcagcacgtgatattgaagcacgtctgaaaaatccggaaaacctgaaactgctgcaagaaggtcacgcactggttggtctgaatccggaagttggtcatgttcgtatgggttttgaagatctgccgtatgcatatgcccgtgttgcacgtgaaggtcgtctgtttcatacccattggaatagccagccgctgggtaattatgatcaggatctgaatattggtgtggtggattgggatagcaccgaagcactgctgtataccctgaaaatggttggttatcagggctattttggcatcgatattaatccggaacgcattccggttgttaaagccattgaaattaacaccaaagtgctgcagattatgaacgaacgcattgaacgtctgccgcatgatcgtattattgagtgttattttgaccctgagaatcatcgtggtgaactggaactgattctggccgaaaatcatcgttaa

SEQ ID NO: 6 - DNA, 1335 bp, Thermotoga Neapolitana
atggcagaatttttcccggaaattccgaaagttcagtttgaaggtaaagaaagcaccaatccgctggcctttaaattctatgatccggaagaaatcattgacggcaaaccgctgaaagatcatctgaaatttagcgttgcattttggcacacctttgtgaatgaaggtcgtgatccgtttggtgatccgaccgcagatcgtccgtggaatcgttataccgatccgatggataaagcatttgcacgtgttgatgcactgtttgaattttgcgaaaaactgaacatcgagtatttctgctttcacgatcgcgatattgcaccggaaggtaaaaccctgcgtgaaaccaacaaaattctggataaagtggtggaacgcatcaaagaacgtatgaaagatagcaatgttaaactgctgtggggcaccgcaaacctgtttagccatccgcgttatatgcatggtgcagcaaccacctgtagcgcagatgtttttgcctatgcagcagcacaggttaaaaaagcactggaaatcaccaaagaactgggtggtgaaggttatgttttttggggtggtcgtgaaggctatgaaacactgctgaataccgatctgggttttgaactggaaaatctggcacgttttctgcgtatggcagttgattatgcaaaacgcattggttttaccggtcagtttctgattgaaccgaaaccgaaagaaccgaccaaacaccagtatgattttgatgttgcaaccgcctatgcctttctgaaaagtcatggtctggatgagtacttcaaatttaacatcgaagcaaatcatgcaaccctggcaggtcatacctttcagcatgaactgcgcatggcacgcattctgggtaaactgggtagcattgatgcaaatcagggtgatctgctgctgggttgggatacagatcagtttccgaccaatgtttatgataccaccctggcaatgtatgaagttattaaagcaggcggttttaccaaaggtggcctgaattttgatgccaaagttcgtcgtgcaagctataaagttgaggacctgtttattggtcatatcgcaggtatggatacctttgcactgggttttaaagttgcctacaaactggttaaagatggcgtgctggataaattcatcgaagaaaaatatcgcagctttcgcgaaggtattggtcgtgatattgttgaaggcaaagtggattttgagaaactggaagagtacatcatcgataaagaaaccattgaactgccgagcggcaaacaagaatatctggaaagcctgattaacagctacatcgtgaaaaccattctggaactgcgttaa

SEQ ID NO: 7 - protein, 388 aa, Streptomyces murinus
MSFQPTPEDRFTFGLWTVGWQGRDPFGDATRPALDPVETVQRLAELGAYGVTFHDDDLIPFGSSDTERESHIKRFRQALDATGMTVPMATTNLFTHPVFKDGGFTANDRDVRRYALRKTIGNIDLAAELGAKTYVAWGGREGAESGGAKDVRDALDRMKEAFDLLGEYVTAQGYDLRFAIEPKPNEPRGDILLPTVGHALAFIERLERPELYGVNPEVGHEQMAGLNFPHGIAQALWAGKLFHIDLNGQSGIKYDQDLRFGAGDLRAAFWLVDLLETAGYEGPRHFDFKPPRTEDFDGVWASAAGCMRNYLILKDRAAAFRADPEVQEALRAARLDQLAQPTAADGLDALLADRAAFEDFDVDAAAARGMAFEHLDQLAMDHLLGARG